European Patent Application EP 4 467 647 A1, published November 27, 2024. Title: RECOMBINANT HUMANIZED COLLAGEN TYPE III ALPHA-1, AND EXPRESSION VECTOR AND USE THEREOF. Applicant: SHANDONG D-NUTRIMEC BIOMEDICAL CO., LTD. The sequence listing filed with the application follows.

SEQUENCE LISTING (3 sequences)

SEQ ID NO: 1 - DNA, 3207 bp, synthetic construct
  source 1..3207: mol_type = other DNA; note = nucleotide sequence of rhCol III a1
caatacgacagttatgatgtaaaaagtggagtggcagttggcggcctggctggttacccggggccagcgggaccaccgggcccgccgggtcccccgggtaccagcggccaccctggaagcccgggcagtccgggttaccagggtccgcccggtgaaccgggtcaagcaggtccgagcggccctcccggtccgccgggtgcaatcggccctagcgggccggctggtaaggacggggagagcggtcgccctggccgtccgggcgagcgcggcctgcccggccctccaggcatcaaaggtccggcgggcattccgggttttccgggtatgaaaggccatcgtggtttcgatggtcgcaatggtgagaaaggggagacgggtgcgcctggtctgaaaggcgaaaacggtctgccgggcgagaacggagcgccgggacctatgggtcctcgtggcgcgccaggtgaacgcggccgcccggggctgccgggggcggctggtgcgcgtggcaacgatggtgcgcgtggctccgatggccaacctggcccgcccggaccacccggcacggcaggttttccgggctcgccgggcgcgaaaggcgaagttggtccggcgggtagcccaggttctaatggcgcgccgggacaacgtggggagccgggtccgcagggccatgcaggggcgcagggcccgccaggaccgccggggatcaacggtagccctggcgggaagggcgagatgggtccggcagggattccgggagccccaggcctgatgggtgcccgcggacctcccggtccggctggggccaatggtgcgcctggactgcgtggtggtgctggcgaaccgggaaagaatggtgcgaaaggcgagccgggcccgcgcggcgaacgtggtgaagctggtatcccgggcgtgccgggtgctaaaggtgaagatggcaaggacgggtcacccggagaaccgggagcgaacggattacctggcgcggcgggagagaggggcgcgccagggtttcgtggcccagcgggtccaaatggaatcccaggcgagaaagggccggctggagaacgtggagcaccgggtccagcgggcccgcgtggtgctgcgggcgaaccggggcgtgacggtgtgccgggcggtccggggatgcgtggcatgcctggttcgccgggaggcccgggttccgatggtaaaccgggcccgccaggcagtcagggggagtccggacgtccgggcccgccgggaccatccggtcctcggggacaaccgggagtgatgggcttcccgggtccgaaaggaaacgatggggcccccggaaaaaacggcgagcgtggtggtccgggcggtccgggaccgcaaggacctccggggaagaacggtgaaaccggtccgcaaggcccaccgggccctacaggacctggaggcgataaaggtgacaccggcccgccgggtcctcaaggtcttcagggtctgccgggtacgggcgggccacctggcgagaatggtaagccgggtgaaccgggccccaagggtgacgccggtgcgccgggtgcacccggcggcaagggcgacgctggcgcaccgggcgaaagaggaccgccaggtttggcgggcgcgcccggactgcgtggcggtgccggtccaccgggtccggaaggtggcaaaggcgctgcggggccacccgggcctccgggcgcggcgggcactccgggtcttcaggggatgccgggcgagcgcggtggtttgggttccccgggtcccaagggtgacaaaggtgaaccgggcggcccaggtgcagacggcgttccgggtaaggacggtccacgtggcccgaccggtcctatcggccctcctggccctgcaggtcagccgggggataagggcgagggtggtgcgccaggactgccgggtatcgcaggtccgcgtggttccccgggcgagcgtggcgaaaccggcccaccgggacctgcgggttttccaggtgcgcctggacaaaacggggagccgggtggtaagggtgagcgtggcgcacctggtgaaaagggggaaggcggccctccgggtgttgcgggccccccggggggctcagggccagctggcccaccgggcccgcagggtgtgaaaggagagagaggttcgccgggaggtcccggtgccgccggtttccctggcgcgcgtggattgccgggaccgcctggtagcaatggtaacccgggcccgccgggaccgagcggttctccgggcaaggacggtcctccgggcccggccggtaacaccggtgcgcccgggtcgccgggtgtcagcggccccaagggcgatgcaggacaaccgggtgagaagggctctccgggtgcgcagggcccgccgggcgctccgggaccgctgggtattgctggaattaccggagcgcgtggactggccggtccgccgggtatgccggggccgcgcggcagcccagggccacagggtgtgaaaggcgagtctggaaagccgggtgcgaacgggctgagcggtgagcgcgggccaccaggcccgcagggtttgccaggccttgccggcaccgcgggagaaccggggcgtgatggaaatccgggttctgatggtctcccgggccgtgatggttccccggggggtaagggcgaccgcggtgagaacggtagcccgggtgcgccaggggcgccgggtcaccctggcccgccgggtcccgtcggtccggcgggcaaaagcggtgaccgtggtgagagcggtccggcggggccggccggcgcgcctggtccggcaggctctcgtggtgcgccaggtcctcaaggccccagaggcgacaagggcgaaaccggagaacgcggtgctgctggcattaaaggtcatcgtggcttcccgggtaacccaggcgcgccaggaagcccgggtccggcagggcagcagggtgccatcggttctccgggcccggcgggtccgcgagggccggttggcccgagcggtccgccgggtaaagacggcaccagcggtcacccgggccccatcggccccccgggtccgcgcggtaatcgtggcgaacgcggatcggaaggttccccgggtcacccaggtcagcctgggccgccgggtccgccgggggctccgggtccgtgttgcggtggcgttggggctgcagcgattgcagggattggtggggagaaagcaggcggtttcgccccttattatggttaa

SEQ ID NO: 2 - DNA, 819 bp, synthetic construct
  source 1..819: mol_type = other DNA; note = DNA of the TEV protease digestion sequence
atgagactgctgaccgccctgttcgcctacttcatcgtggccctgatcctggccttcagcgtgtccgccaagagcatgcaccaccaccatcaccatcatcacatgagcaagggcgaggaactgttcaccggcgtggtgcccatcctggtggaactggacggcgacgtgaacggccacaagttctctgtgcggggcgagggcgagggggacgccacaaatggcaagctgaccctgaagttcatctgcaccaccggaaagctgcccgtgccctggcctaccctggtcacaaccctgacctacggcgtgcagtgcttcagcagataccccgaccacatgaagcggcacgatttcttcaagagcgccatgcccgagggctacgtgcaagaacggaccatcagcttcaaggacgacggcacctacaagaccagagccgaagtgaagttcgagggcgacaccctggtcaaccggatcgagctgaagggcatcgacttcaaagaggacggcaacatcctgggccacaagctggaatacaacttcaacagccacaacgtgtacatcaccgccgacaagcagaagaacggcatcaaggccaacttcaagatccggcacaacgtggaagatggcagcgtgcagctggccgaccactaccagcagaacacccccatcggcgacggccccgtgctgctgcccgacaatcactacctgagcacccagagcgtgctgagcaaggaccccaacgagaagcgggaccacatggtgctgctggaatttgtgaccgccgctggcatcacccacggcgagaacctgtacttccaaggg

SEQ ID NO: 3 - protein, 1320 aa, synthetic construct
  source 1..1320: note = amino acid sequence of the rhCol III a1 fusion protein
KSMHHHHHHHHMSKGEELFTGVVPILVELDGDVNGHKFSVRGEGEGDATNGKLTLKFICTTGKLPVPWPTLVTTLTYGVQCFSRYPDHMKRHDFFKSAMPEGYVQERTISFKDDGTYKTRAEVKFEGDTLVNRIELKGIDFKEDGNILGHKLEYNFNSHNVYITADKQKNGIKANFKIRHNVEDGSVQLADHYQQNTPIGDGPVLLPDNHYLSTQSVLSKDPNEKRDHMVLLEFVTAAGITHGENLYFQGGSQYDSYDVKSGVAVGGLAGYPGPAGPPGPPGPPGTSGHPGSPGSPGYQGPPGEPGQAGPSGPPGPPGAIGPSGPAGKDGESGRPGRPGERGLPGPPGIKGPAGIPGFPGMKGHRGFDGRNGEKGETGAPGLKGENGLPGENGAPGPMGPRGAPGERGRPGLPGAAGARGNDGARGSDGQPGPPGPPGTAGFPGSPGAKGEVGPAGSPGSNGAPGQRGEPGPQGHAGAQGPPGPPGINGSPGGKGEMGPAGIPGAPGLMGARGPPGPAGANGAPGLRGGAGEPGKNGAKGEPGPRGERGEAGIPGVPGAKGEDGKDGSPGEPGANGLPGAAGERGAPGFRGPAGPNGIPGEKGPAGERGAPGPAGPRGAAGEPGRDGVPGGPGMRGMPGSPGGPGSDGKPGPPGSQGESGRPGPPGPSGPRGQPGVMGFPGPKGNDGAPGKNGERGGPGGPGPQGPPGKNGETGPQGPPGPTGPGGDKGDTGPPGPQGLQGLPGTGGPPGENGKPGEPGPKGDAGAPGAPGGKGDAGAPGERGPPGLAGAPGLRGGAGPPGPEGGKGAAGPPGPPGAAGTPGLQGMPGERGGLGSPGPKGDKGEPGGPGADGVPGKDGPRGPTGPIGPPGPAGQPGDKGEGGAPGLPGIAGPRGSPGERGETGPPGPAGFPGAPGQNGEPGGKGERGAPGEKGEGGPPGVAGPPGGSGPAGPPGPQGVKGERGSPGGPGAAGFPGARGLPGPPGSNGNPGPPGPSGSPGKDGPPGPAGNTGAPGSPGVSGPKGDAGQPGEKGSPGAQGPPGAPGPLGIAGITGARGLAGPPGMPGPRGSPGPQGVKGESGKPGANGLSGERGPPGPQGLPGLAGTAGEPGRDGNPGSDGLPGRDGSPGGKGDRGENGSPGAPGAPGHPGPPGPVGPAGKSGDRGESGPAGPAGAPGPAGSRGAPGPQGPRGDKGETGERGAAGIKGHRGFPGNPGAPGSPGPAGQQGAIGSPGPAGPRGPVGPSGPPGKDGTSGHPGPIGPPGPRGNRGERGSEGSPGHPGQPGPPGPPGAPGPCCGGVGAAAIAGIGGEKAGGFAPYYG